European Patent Application EP 4 715 051 A1, published March 25, 2026. Title: 小核酸在制备治疗猫传染性腹膜炎药物中的应用. Applicant: 南京晖丽生物科技有限公司. The sequence listing filed with the application follows.

SEQUENCE LISTING (55 sequences)

SEQ ID NO: 1 - RNA, 21 nt, synthetic construct
  source 1..21: mol_type = other RNA; note = Small RNA
ccgccgggatattgtgttcgg

SEQ ID NO: 2 - RNA, 25 nt, synthetic construct
  source 1..25: mol_type = other RNA; note = Small RNA
taggccgggggactgtactgatgtt

SEQ ID NO: 3 - RNA, 24 nt, synthetic construct
  source 1..24: mol_type = other RNA; note = Small RNA
ccagccgggggagacatcctcggg

SEQ ID NO: 4 - RNA, 25 nt, synthetic construct
  source 1..25: mol_type = other RNA; note = Small RNA
atcggccgggggttccctatcggca

SEQ ID NO: 5 - RNA, 25 nt, synthetic construct
  source 1..25: mol_type = other RNA; note = Small RNA
caggccgggggatgctcgcaaagct

SEQ ID NO: 6 - RNA, 24 nt, synthetic construct
  source 1..24: mol_type = other RNA; note = Small RNA
gcagccgggggcgaacatcgcacg

SEQ ID NO: 7 - RNA, 26 nt, synthetic construct
  source 1..26: mol_type = other RNA; note = Small RNA
atgccgggggcgacaaagaatctttt

SEQ ID NO: 8 - RNA, 25 nt, synthetic construct
  source 1..25: mol_type = other RNA; note = Small RNA
acgccgggggataaatccacgcctc

SEQ ID NO: 9 - RNA, 20 nt, synthetic construct
  source 1..20: mol_type = other RNA; note = Small RNA
aagccggggcgtcttctccc

SEQ ID NO: 10 - RNA, 22 nt, synthetic construct
  source 1..22: mol_type = other RNA; note = Small RNA
ttggccgggggcctccgcgcgg

SEQ ID NO: 11 - RNA, 26 nt, synthetic construct
  source 1..26: mol_type = other RNA; note = Small RNA
taggccgggggctggtctgggtttat

SEQ ID NO: 12 - RNA, 26 nt, synthetic construct
  source 1..26: mol_type = other RNA; note = Small RNA
gtggccgggggcgagtatccctccgc

SEQ ID NO: 13 - RNA, 25 nt, synthetic construct
  source 1..25: mol_type = other RNA; note = Small RNA
cgcgccgggggccagcttaatctcc

SEQ ID NO: 14 - RNA, 26 nt, synthetic construct
  source 1..26: mol_type = other RNA; note = Small RNA
tcggccgggggcgagtgaccgcaatt

SEQ ID NO: 15 - RNA, 25 nt, synthetic construct
  source 1..25: mol_type = other RNA; note = Small RNA
acgccgggggatattccgaacctgc

SEQ ID NO: 16 - RNA, 25 nt, synthetic construct
  source 1..25: mol_type = other RNA; note = Small RNA
gctgccgggggggtgactgtgcata

SEQ ID NO: 17 - RNA, 24 nt, synthetic construct
  source 1..24: mol_type = other RNA; note = Small RNA
ccagccgggggcgccccggtcgat

SEQ ID NO: 18 - RNA, 24 nt, synthetic construct
  source 1..24: mol_type = other RNA; note = Small RNA
cggccgggggctccaccggagata

SEQ ID NO: 19 - RNA, 26 nt, synthetic construct
  source 1..26: mol_type = other RNA; note = Small RNA
ggccgggggactttcggagagcgtga

SEQ ID NO: 20 - RNA, 20 nt, synthetic construct
  source 1..20: mol_type = other RNA; note = Small RNA
gggccggggtatgttttcgg

SEQ ID NO: 21 - RNA, 24 nt, synthetic construct
  source 1..24: mol_type = other RNA; note = Small RNA
tggccgggggctgccccaagactg

SEQ ID NO: 22 - RNA, 22 nt, synthetic construct
  source 1..22: mol_type = other RNA; note = Small RNA
agccggggggagggtctgcaag

SEQ ID NO: 23 - RNA, 25 nt, synthetic construct
  source 1..25: mol_type = other RNA; note = Small RNA
ctagccgggggagctggtcatactc

SEQ ID NO: 24 - RNA, 26 nt, synthetic construct
  source 1..26: mol_type = other RNA; note = Small RNA
ctccgccgggggaatccctgcggata

SEQ ID NO: 25 - RNA, 22 nt, synthetic construct
  source 1..22: mol_type = other RNA; note = Small RNA
tggccgggggagttgattaata

SEQ ID NO: 26 - RNA, 24 nt, synthetic construct
  source 1..24: mol_type = other RNA; note = Small RNA
cagccgggggcagcttaggcgaca

SEQ ID NO: 27 - RNA, 24 nt, synthetic construct
  source 1..24: mol_type = other RNA; note = Small RNA
tcgccgggggtatctaacgtgttc

SEQ ID NO: 28 - RNA, 21 nt, synthetic construct
  source 1..21: mol_type = other RNA; note = Small RNA
tggccggggggggggtcggtc

SEQ ID NO: 29 - RNA, 23 nt, synthetic construct
  source 1..23: mol_type = other RNA; note = Small RNA
accgccgggggcaatacaaagag

SEQ ID NO: 30 - RNA, 26 nt, synthetic construct
  source 1..26: mol_type = other RNA; note = Small RNA
ttggccgggggaggcctagttggaat

SEQ ID NO: 31 - RNA, 26 nt, synthetic construct
  source 1..26: mol_type = other RNA; note = Small RNA
gcgccgggggttcgacagggaaaaga

SEQ ID NO: 32 - RNA, 25 nt, synthetic construct
  source 1..25: mol_type = other RNA; note = Small RNA
atgccggggggcagttagaagcgat

SEQ ID NO: 33 - RNA, 21 nt, synthetic construct
  source 1..21: mol_type = other RNA; note = Small RNA
tggccgggggatacgtgcgta

SEQ ID NO: 34 - RNA, 25 nt, synthetic construct
  source 1..25: mol_type = other RNA; note = Small RNA
gggccgggggcatagtactctcccg

SEQ ID NO: 35 - RNA, 22 nt, synthetic construct
  source 1..22: mol_type = other RNA; note = Small RNA
ccgccgggggataaagagcaaa

SEQ ID NO: 36 - RNA, 24 nt, synthetic construct
  source 1..24: mol_type = other RNA; note = Small RNA
gccgggggcctcaaatcctcgcca

SEQ ID NO: 37 - RNA, 19 nt, synthetic construct
  source 1..19: mol_type = other RNA; note = Small RNA
cgccgggggaacatcctta

SEQ ID NO: 38 - RNA, 21 nt, synthetic construct
  source 1..21: mol_type = other RNA; note = Small RNA
cgccgggggcccggctcttcc

SEQ ID NO: 39 - RNA, 23 nt, synthetic construct
  source 1..23: mol_type = other RNA; note = Small RNA
tcgccgggggttacttcagatta

SEQ ID NO: 40 - RNA, 25 nt, synthetic construct
  source 1..25: mol_type = other RNA; note = Small RNA
ttagccgggaattcagcacgaccaa

SEQ ID NO: 41 - RNA, 22 nt, synthetic construct
  source 1..22: mol_type = other RNA; note = Small RNA
atgccgggggctgtataccgat

SEQ ID NO: 42 - RNA, 26 nt, synthetic construct
  source 1..26: mol_type = other RNA; note = Small RNA
aaggccggggggaaggaaacgctcta

SEQ ID NO: 43 - RNA, 26 nt, synthetic construct
  source 1..26: mol_type = other RNA; note = Small RNA
gtgccgggggggtacgtcacgactat

SEQ ID NO: 44 - RNA, 24 nt, synthetic construct
  source 1..24: mol_type = other RNA; note = Small RNA
acgccgggggcgtggtactaccat

SEQ ID NO: 45 - RNA, 25 nt, synthetic construct
  source 1..25: mol_type = other RNA; note = Small RNA
gatgccgggggacgttgctgtttcc

SEQ ID NO: 46 - RNA, 23 nt, synthetic construct
  source 1..23: mol_type = other RNA; note = Small RNA
gagccgggggtatggcggcgatg

SEQ ID NO: 47 - RNA, 24 nt, synthetic construct
  source 1..24: mol_type = other RNA; note = Small RNA
gagccggggggatcaactaggttt

SEQ ID NO: 48 - RNA, 24 nt, synthetic construct
  source 1..24: mol_type = other RNA; note = Small RNA
tgccgggggcggtctatttcggga

SEQ ID NO: 49 - RNA, 24 nt, synthetic construct
  source 1..24: mol_type = other RNA; note = Small RNA
cagccgggggctcaggccatcccc

SEQ ID NO: 50 - RNA, 23 nt, synthetic construct
  source 1..23: mol_type = other RNA; note = Small RNA
ggccgggggccaggcgtcccccc

SEQ ID NO: 51 - RNA, 24 nt, synthetic construct
  source 1..24: mol_type = other RNA; note = Small RNA
ttgccgggggaagactcctatccg

SEQ ID NO: 52 - RNA, 27 nt, synthetic construct
  source 1..27: mol_type = other RNA; note = Small RNA
atggccggggggagggatgtcttactc

SEQ ID NO: 53 - RNA, 25 nt, synthetic construct
  source 1..25: mol_type = other RNA; note = Small RNA
cggccggggggtcaaagcttcgtgt

SEQ ID NO: 54 - RNA, 20 nt, Populus euphratica
  source 1..20: mol_type = genomic RNA
cggccgggggacgggctggg

SEQ ID NO: 55 - DNA, 21 bp, synthetic construct
  source 1..21: mol_type = other DNA; note = DNA sequence of small RNA 1
ccgccgggatattgtgttcgg